European Patent Application EP 4 509 136 A1, published February 19, 2025. Title: Fusion protein and use thereof. Applicant: SHANXI JINBO BIO-PHARMACEUTICAL CO., LTD. Application EP. The sequence listing filed with the application follows.

SEQUENCE LISTING (10 sequences)

SEQ ID NO: 1 - protein, 30 aa, synthetic construct
GERGAPGFRGPAGPNGIPGEKGPAGERGAP

SEQ ID NO: 2 - protein, 9 aa, synthetic construct
  REGION 1..9: note = C
GAPGPCCGG

SEQ ID NO: 3 - protein, 489 aa, synthetic construct
  REGION 1..489: note = tri region
GERGAPGFRGPAGPNGIPGEKGPAGERGAPGERGAPGFRGPAGPNGIPGEKGPAGERGAPGERGAPGFRGPAGPNGIPGEKGPAGERGAPGERGAPGFRGPAGPNGIPGEKGPAGERGAPGERGAPGFRGPAGPNGIPGEKGPAGERGAPGERGAPGFRGPAGPNGIPGEKGPAGERGAPGERGAPGFRGPAGPNGIPGEKGPAGERGAPGERGAPGFRGPAGPNGIPGEKGPAGERGAPGERGAPGFRGPAGPNGIPGEKGPAGERGAPGERGAPGFRGPAGPNGIPGEKGPAGERGAPGERGAPGFRGPAGPNGIPGEKGPAGERGAPGERGAPGFRGPAGPNGIPGEKGPAGERGAPGERGAPGFRGPAGPNGIPGEKGPAGERGAPGERGAPGFRGPAGPNGIPGEKGPAGERGAPGERGAPGFRGPAGPNGIPGEKGPAGERGAPGERGAPGFRGPAGPNGIPGEKGPAGERGAPGAPGPCCGG

SEQ ID NO: 4 - protein, 214 aa, synthetic construct
  REGION 1..214: note = SARS-CoV-2 RBD protein
RVQPTESIVRFPNITNLCPFGEVFNATRFASVYAWNRKRISNCVADYSVLYNSASFSTFKCYGVSPTKLNDLCFTNVYADSFVIRGDEVRQIAPGQTGKIADYNYKLPDDFTGCVIAWNSNNLDSKVGGNYNYRYRLFRKSNLKPFERDISTEIYQAGSKPCNGVEGFNCYFPLQSYGFQPTNGVGYQPYRVVVLSFELLHAPATVCGPKKSTN

SEQ ID NO: 5 - protein, 723 aa, synthetic construct
  REGION 1..723: note = fusion protein without his tag
GERGAPGFRGPAGPNGIPGEKGPAGERGAPGERGAPGFRGPAGPNGIPGEKGPAGERGAPGERGAPGFRGPAGPNGIPGEKGPAGERGAPGERGAPGFRGPAGPNGIPGEKGPAGERGAPGERGAPGFRGPAGPNGIPGEKGPAGERGAPGERGAPGFRGPAGPNGIPGEKGPAGERGAPGERGAPGFRGPAGPNGIPGEKGPAGERGAPGERGAPGFRGPAGPNGIPGEKGPAGERGAPGERGAPGFRGPAGPNGIPGEKGPAGERGAPGERGAPGFRGPAGPNGIPGEKGPAGERGAPGERGAPGFRGPAGPNGIPGEKGPAGERGAPGERGAPGFRGPAGPNGIPGEKGPAGERGAPGERGAPGFRGPAGPNGIPGEKGPAGERGAPGERGAPGFRGPAGPNGIPGEKGPAGERGAPGERGAPGFRGPAGPNGIPGEKGPAGERGAPGERGAPGFRGPAGPNGIPGEKGPAGERGAPGAPGPCCGGGGGGSGGGGSGGGGSGGGGSRVQPTESIVRFPNITNLCPFGEVFNATRFASVYAWNRKRISNCVADYSVLYNSASFSTFKCYGVSPTKLNDLCFTNVYADSFVIRGDEVRQIAPGQTGKIADYNYKLPDDFTGCVIAWNSNNLDSKVGGNYNYRYRLFRKSNLKPFERDISTEIYQAGSKPCNGVEGFNCYFPLQSYGFQPTNGVGYQPYRVVVLSFELLHAPATVCGPKKSTN

SEQ ID NO: 6 - protein, 731 aa, synthetic construct
  REGION 1..731: note = His
GERGAPGFRGPAGPNGIPGEKGPAGERGAPGERGAPGFRGPAGPNGIPGEKGPAGERGAPGERGAPGFRGPAGPNGIPGEKGPAGERGAPGERGAPGFRGPAGPNGIPGEKGPAGERGAPGERGAPGFRGPAGPNGIPGEKGPAGERGAPGERGAPGFRGPAGPNGIPGEKGPAGERGAPGERGAPGFRGPAGPNGIPGEKGPAGERGAPGERGAPGFRGPAGPNGIPGEKGPAGERGAPGERGAPGFRGPAGPNGIPGEKGPAGERGAPGERGAPGFRGPAGPNGIPGEKGPAGERGAPGERGAPGFRGPAGPNGIPGEKGPAGERGAPGERGAPGFRGPAGPNGIPGEKGPAGERGAPGERGAPGFRGPAGPNGIPGEKGPAGERGAPGERGAPGFRGPAGPNGIPGEKGPAGERGAPGERGAPGFRGPAGPNGIPGEKGPAGERGAPGERGAPGFRGPAGPNGIPGEKGPAGERGAPGAPGPCCGGGGGGSGGGGSGGGGSGGGGSRVQPTESIVRFPNITNLCPFGEVFNATRFASVYAWNRKRISNCVADYSVLYNSASFSTFKCYGVSPTKLNDLCFTNVYADSFVIRGDEVRQIAPGQTGKIADYNYKLPDDFTGCVIAWNSNNLDSKVGGNYNYRYRLFRKSNLKPFERDISTEIYQAGSKPCNGVEGFNCYFPLQSYGFQPTNGVGYQPYRVVVLSFELLHAPATVCGPKKSTNHHHHHHHH

SEQ ID NO: 7 - DNA, 2196 bp, synthetic construct
  misc_feature 1..2196: note = nucleic acid encoding the fusion protein
  source 1..2196: mol_type = other DNA
ggagaacgtggagcccccggattcagaggaccagccggccccaacggaatccctggtgagaagggccctgccggcgaaaggggcgccccgggcgagagaggagcccctggcttccggggcccggccgggcctaatggcatccctggcgagaagggccctgctggagaacggggcgcccccggcgagcgcggagctcccggcttccggggcccagccgggcctaacggcatccctggcgagaagggccctgccggcgagaggggcgctcctggggagagaggcgcccctggcttcagaggacccgccggtcctaatggaatccccggcgagaagggccctgccggcgaaagaggcgcccctggagagagaggcgctcctggatttagaggtccagccggtcccaacggaatccctggagagaaggggcccgctggcgaaagaggagcccctggcgaaagaggcgcccccggatttagaggacctgcaggccctaatggaatccctggcgagaagggccctgccggagaacggggcgcccctggcgagagaggtgcccctggctttagaggccccgctggccccaacggcatccctggggagaaaggcccggccggcgaacggggagccccgggcgagaggggcgccccaggattccggggccctgctggccccaacggcattcctggcgaaaaaggccctgccggggagcggggcgcccctggcgaaagaggcgctcctggtttccggggccctgctgggcctaacggcatccccggcgaaaagggcccagccggggagagaggagcccctggcgagcggggagctcctggcttcagaggccctgccggccctaacggcatccccggcgaaaaaggccccgccggtgaaagaggggcgcccggtgaaagaggcgcccctggcttccggggccctgccggcccaaatggtatccctggagaaaagggccctgcaggagagcgtggcgcccctggcgaacgcggcgcccctggctttagaggcccagcaggccctaacggcatccctggcgagaaaggacccgctggtgaaagaggcgccccaggcgagagaggggctcctggcttcagaggcccagccggcccaaacggcatccctggcgagaagggccccgccggcgaacggggcgccccgggcgagagaggagcccccggtttccggggtcccgccggccctaatggcatccccggcgagaaaggacctgccggcgagcggggcgctcctggagagcggggcgcccctggcttccggggccctgctggccctaacggaatccctggcgaaaaaggccctgccggcgagagaggcgcccccggcgagagaggggccccaggcttccggggacctgccggccctaacggcatccctggcgagaagggccctgctggcgaaagaggcgcccccggagcgcctggcccctgttgcggcggaggaggaggtggatctggcggcggaggcagcggaggcggcggctctgggggcggcggctccagagtgcagcctacagagagcatcgtgcggttccccaacatcaccaacctgtgtcctttcggtgaggtgttcaacgctaccagattcgccagcgtgtacgcctggaatagaaagagaatcagcaattgcgtggccgactacagcgtgctgtacaacagcgcctctttcagcaccttcaagtgctatggcgtgtcccctaccaagctgaacgacctgtgcttcaccaacgtgtacgccgacagcttcgtgatcagaggcgatgaggtgagacagatcgcccctggccagaccggcaagatcgccgattacaactacaagctgcctgacgacttcaccggttgtgtgatcgcctggaacagcaacaacctggacagcaaggtgggcggaaattacaactacagatacagactgttcagaaagtccaacctcaagcccttcgagagagatatctctacagaaatctaccaggccggatctaagccttgcaacggcgtggaaggctttaactgctacttccctctgcagagctacggctttcagcccaccaacggcgttggttatcaaccttacagagtcgtggtcctgagctttgagctgctgcacgcccctgctacagtgtgcggccccaagaagagcacaaaccaccaccaccaccaccaccaccattga

SEQ ID NO: 8 - protein, 20 aa, synthetic construct
  REGION 1..20: note = linker
GGGGSGGGGSGGGGSGGGGS

SEQ ID NO: 9 - protein, 843 aa, synthetic construct
GERGAPGFRGPAGPNGIPGEKGPAGERGAPGERGAPGFRGPAGPNGIPGEKGPAGERGAPGERGAPGFRGPAGPNGIPGEKGPAGERGAPGERGAPGFRGPAGPNGIPGEKGPAGERGAPGERGAPGFRGPAGPNGIPGEKGPAGERGAPGERGAPGFRGPAGPNGIPGEKGPAGERGAPGERGAPGFRGPAGPNGIPGEKGPAGERGAPGERGAPGFRGPAGPNGIPGEKGPAGERGAPGERGAPGFRGPAGPNGIPGEKGPAGERGAPGERGAPGFRGPAGPNGIPGEKGPAGERGAPGERGAPGFRGPAGPNGIPGEKGPAGERGAPGERGAPGFRGPAGPNGIPGEKGPAGERGAPGERGAPGFRGPAGPNGIPGEKGPAGERGAPGERGAPGFRGPAGPNGIPGEKGPAGERGAPGERGAPGFRGPAGPNGIPGEKGPAGERGAPGERGAPGFRGPAGPNGIPGEKGPAGERGAPGAPGPCCGGGGGGSGGGGSGGGGSGGGGSDTICIGYHANNSTDTVDTIFEKNVAVTHSVNLLEDRHNGKLCKLKGIAPLQLGKCNIIGWLLGNPECDSLLPARSWSYIVETPNSENGACYPGDFIDYEELREQLSSVSSLERFEIFPKESSWPNHTFNGVTASCSHRGKSSFYRNLLWLTKKGDSYPKLTNSYVNNKGKEVLVLWGVHHPSSSDEQQSLYSNGNAYVSVASSNYNRRFTPEIAARPKVKDQHGRMNYYWTLLEPGDTIIFEATGNLIAPWYAFALSRGFESGIITSNASMHECNTKCQTPQGSINSNLPFQNIHPVTIGECPKYVRSTKLRMVTGLRNIPSIQYRHHHHHHHH

SEQ ID NO: 10 - protein, 326 aa, synthetic construct
DTICIGYHANNSTDTVDTIFEKNVAVTHSVNLLEDRHNGKLCKLKGIAPLQLGKCNIIGWLLGNPECDSLLPARSWSYIVETPNSENGACYPGDFIDYEELREQLSSVSSLERFEIFPKESSWPNHTFNGVTASCSHRGKSSFYRNLLWLTKKGDSYPKLTNSYVNNKGKEVLVLWGVHHPSSSDEQQSLYSNGNAYVSVASSNYNRRFTPEIAARPKVKDQHGRMNYYWTLLEPGDTIIFEATGNLIAPWYAFALSRGFESGIITSNASMHECNTKCQTPQGSINSNLPFQNIHPVTIGECPKYVRSTKLRMVTGLRNIPSIQYR